European Patent Application EP 4 563 155 A1, published June 4, 2025. Title: Composition for preventing, ameliorating or treating respiratory disease comprising zinc salt and cyclo-hispro as active ingredient. Applicant: NOVMETAPHARMA CO., LTD. The sequence listing filed with the application follows.

SEQUENCE LISTING (10 sequences)

SEQ ID NO: 1 - DNA, 20 bp, synthetic construct
  misc_feature 1..20: note = IL-4 forward primer
  source 1..20: mol_type = other DNA
tcggcattttgaacgaggtc

SEQ ID NO: 2 - DNA, 20 bp, synthetic construct
  misc_feature 1..20: note = IL-4 reverse primer
  source 1..20: mol_type = other DNA
cgttgctgtgaggacgtttg

SEQ ID NO: 3 - DNA, 21 bp, synthetic construct
  misc_feature 1..21: note = IL-13 forward primer
  source 1..21: mol_type = other DNA
ccatctacaggacccagagga

SEQ ID NO: 4 - DNA, 20 bp, synthetic construct
  misc_feature 1..20: note = IL-13 reverse primer
  source 1..20: mol_type = other DNA
ttttggtatcggggaggctg

SEQ ID NO: 5 - DNA, 19 bp, synthetic construct
  misc_feature 1..19: note = IL-17a forward primer
  source 1..19: mol_type = other DNA
cctcacacgaggcacaagt

SEQ ID NO: 6 - DNA, 20 bp, synthetic construct
  misc_feature 1..20: note = IL-17a reverse primer
  source 1..20: mol_type = other DNA
tgaagctctccctggactca

SEQ ID NO: 7 - DNA, 21 bp, synthetic construct
  misc_feature 1..21: note = Muc5ac forward primer
  source 1..21: mol_type = other DNA
tgtgcctgcctgtacaatggg

SEQ ID NO: 8 - DNA, 23 bp, synthetic construct
  misc_feature 1..23: note = Muc5ac reverse primer
  source 1..23: mol_type = other DNA
catgtgttggtgcagtcagtaga

SEQ ID NO: 9 - DNA, 20 bp, synthetic construct
  misc_feature 1..20: note = hprt forward primer
  source 1..20: mol_type = other DNA
aaatgtcagttgctgcgtcc

SEQ ID NO: 10 - DNA, 20 bp, synthetic construct
  misc_feature 1..20: note = hprt reverse primer
  source 1..20: mol_type = other DNA
tctaccagagggtaggctgg